European Patent Application EP 4 122 464 A1, published January 25, 2023. Title: METHODS OF TREATING LIVER DISEASE. Applicant: Gilead Sciences, Inc. The sequence listing filed with the application follows.

SEQUENCE LISTING (8 sequences)

SEQ ID NO: 1 - DNA, 100 bp, Artificial Sequence
  Synthetic
aagcctctgtggatatgcccacaagtcccagaaccgcagtgaagagtttctcatcacgggccgcctaaggaacggaaatttgcacatcagtgcctgcagc

SEQ ID NO: 2 - DNA, 100 bp, Artificial Sequence
  Synthetic
caatggtgagacgtggaaacccgaggtatgcttgatctgtatctgccacaatggcacggctgtgtgcgatgacgtgcaatgcaatgaagaactggactgt

SEQ ID NO: 3 - DNA, 100 bp, Artificial Sequence
  Synthetic
catacgcctgcagagttaagcatgccagtatggccgagcccaagaccgtctactgggatcgagacatgtgatcaagcatcatgatgctctgaagattcat

SEQ ID NO: 4 - DNA, 100 bp, Artificial Sequence
  Synthetic
tgctgaggcggcgagggagagcgttgggcttacctcactgctttccggagcggtagcacctcctccgccggcttcctcctcagaccgctttttgccgcga

SEQ ID NO: 5 - DNA, 100 bp, Artificial Sequence
  Synthetic
ccggcattctgcacgcttcaaaagcgcacgtctgccgcgctgttctcctcttcctcatctccgggcctttcgacctcacggtgttgccaaaatgtcgctt

SEQ ID NO: 6 - DNA, 100 bp, Artificial Sequence
  Synthetic
atgggatccctccaccctatgacaagaaaaagcggatggtggtccctgctgctctcaaggttgttcggctgaagcctaccagaaagtttgcttacctggg

SEQ ID NO: 7 - DNA, 100 bp, Artificial Sequence
  Synthetic
ggcagcctgacagtgggatctcctccattcgttcttttaagaccatccttcctgctgccgcccaggatgtctattaccgggatgagattggtaatgtttc

SEQ ID NO: 8 - DNA, 101 bp, Artificial Sequence
  Synthetic
gatgctcacaagggacgcaaaaacgaaggagtgattgaatttgtgtcttactctgatatgaaaagagctttggaaaagctggacggaactgaagtcaacgg